European Patent Application EP 4 134 092 A1, published February 15, 2023. Title: Novel Antimicrobial Peptides or Peptide Analogues And Use Thereof. Applicant: CAMP Therapeutics Inc. The sequence listing filed with the application follows.

SEQUENCE LISTING (67 sequences)

SEQ ID NO: 1 - protein, 15 aa, Artificial Sequence
  synthetic peptide
KKLLKLLKKPLKLLK

SEQ ID NO: 2 - protein, 15 aa, Artificial Sequence
  synthetic peptide
AKLLKLLKKPLKLLK

SEQ ID NO: 3 - protein, 15 aa, Artificial Sequence
  synthetic peptide
KALLKLLKKPLKLLK

SEQ ID NO: 4 - protein, 15 aa, Artificial Sequence
  synthetic peptide
KKALKLLKKPLKLLK

SEQ ID NO: 5 - protein, 15 aa, Artificial Sequence
  synthetic peptide
KKLAKLLKKPLKLLK

SEQ ID NO: 6 - protein, 15 aa, Artificial Sequence
  synthetic peptide
KKLLALLKKPLKLLK

SEQ ID NO: 7 - protein, 15 aa, Artificial Sequence
  synthetic peptide
KKLLKALKKPLKLLK

SEQ ID NO: 8 - protein, 15 aa, Artificial Sequence
  synthetic peptide
KKLLKLAKKPLKLLK

SEQ ID NO: 9 - protein, 15 aa, Artificial Sequence
  synthetic peptide
KKLLKLLAKPLKLLK

SEQ ID NO: 10 - protein, 15 aa, Artificial Sequence
  synthetic peptide
KKLLKLLKAPLKLLK

SEQ ID NO: 11 - protein, 15 aa, Artificial Sequence
  synthetic peptide
KKLLKLLKKPAKLLK

SEQ ID NO: 12 - protein, 15 aa, Artificial Sequence
  synthetic peptide
KKLLKLLKKPLALLK

SEQ ID NO: 13 - protein, 15 aa, Artificial Sequence
  synthetic peptide
KKLLKLLKKPLKALK

SEQ ID NO: 14 - protein, 15 aa, Artificial Sequence
  synthetic peptide
KKLLKLLKKPLKLAK

SEQ ID NO: 15 - protein, 15 aa, Artificial Sequence
  synthetic peptide
KKLLKLLKKPLKLLA

SEQ ID NO: 16 - protein, 15 aa, Artificial Sequence
  synthetic peptide
KKALKLAKKPLKLLK

SEQ ID NO: 17 - protein, 15 aa, Artificial Sequence
  synthetic peptide
KKVLKLVKKPLKLLK

SEQ ID NO: 18 - protein, 15 aa, Artificial Sequence
  synthetic peptide
  MISC_FEATURE (1): N-terminal is lipidated by OctA(octanoic acid)
KKALKLAKKPLKLLK

SEQ ID NO: 19 - protein, 15 aa, Artificial Sequence
  synthetic peptide
  MISC_FEATURE (1): N-terminal is lipidated by HexA(hexanoic acid)
KKLLKLLKKPLKLLK

SEQ ID NO: 20 - protein, 15 aa, Artificial Sequence
  synthetic peptide
  MISC_FEATURE (1): N-terminal is lipidated by HexA
KKLLKLAKKPLKLLK

SEQ ID NO: 21 - protein, 15 aa, Artificial Sequence
  synthetic peptide
  MISC_FEATURE (1): N-terminal is lipidated by HexA
KKLLKLVKKPLKLLK

SEQ ID NO: 22 - protein, 15 aa, Artificial Sequence
  synthetic peptide
  MISC_FEATURE (1): N-terminal is lipidated by HexA
KKVLKLVKKPLKLLK

SEQ ID NO: 23 - protein, 15 aa, Artificial Sequence
  synthetic peptide
  MISC_FEATURE (1): N-terminal is lipidated by HexA
KKALKLAKKPLKLLK

SEQ ID NO: 24 - protein, 15 aa, Artificial Sequence
  synthetic peptide
  MISC_FEATURE (1): N-terminal is lipidated by OctA
KKLLKLLKKPLKLLK

SEQ ID NO: 25 - protein, 15 aa, Artificial Sequence
  synthetic peptide
  MISC_FEATURE (1): N-terminal is lipidated by DecA(decanoic acid)
KKALKLAKKPLKLLK

SEQ ID NO: 26 - protein, 15 aa, Artificial Sequence
  synthetic peptide
  MISC_FEATURE (1): N-terminal is lipidated by LauA(lauric acid)
KKALKLAKKPLKLLK

SEQ ID NO: 27 - protein, 15 aa, Artificial Sequence
  synthetic peptide
  MISC_FEATURE (1): N-terminal is lipidated by OctA
  MISC_FEATURE (1)..(2): X is Dab(diaminobutyric acid)
  MISC_FEATURE (5): X is Dab
  MISC_FEATURE (8)..(9): X is Dab
  MISC_FEATURE (12): X is Dab
  MISC_FEATURE (15): X is Dab
XXALXLAXXPLXLLX

SEQ ID NO: 28 - protein, 15 aa, Artificial Sequence
  synthetic peptide
  MISC_FEATURE (1): N-terminal is lipidated by LauA
  MISC_FEATURE (1)..(2): X is Dab
  MISC_FEATURE (5): X is Dab
  MISC_FEATURE (8)..(9): X is Dab
  MISC_FEATURE (12): X is Dab
  MISC_FEATURE (15): X is Dab
XXALXLAXXPLXLLX

SEQ ID NO: 29 - protein, 15 aa, Artificial Sequence
  synthetic peptide
  MISC_FEATURE (1): N-terminal is lipidated by OctA
  MISC_FEATURE (1)..(2): X is Dab
  MISC_FEATURE (4): X is Hdf
  MISC_FEATURE (5): X is Dab
  MISC_FEATURE (6)..(7): X is Hdf
  MISC_FEATURE (8)..(9): X is Dab
  MISC_FEATURE (12): X is Dab
  MISC_FEATURE (15): X is Dab
XXAXXXXXXPLXLLX

SEQ ID NO: 30 - protein, 15 aa, Artificial Sequence
  synthetic peptide
  MISC_FEATURE (1): N-terminal is lipidated by OctA
  MISC_FEATURE (1)..(2): X is Dab
  MISC_FEATURE (4): X is Hdf
  MISC_FEATURE (5): X is Dab
  MISC_FEATURE (6)..(7): X is Hdf
  MISC_FEATURE (8)..(9): X is Dab
  MISC_FEATURE (12): X is Dab
  MISC_FEATURE (15): X is Dab
XXFXXXXXXPLXLLX

SEQ ID NO: 31 - protein, 15 aa, Artificial Sequence
  synthetic peptide
  MISC_FEATURE (1): N-terminal is lipidated by OctA
  MISC_FEATURE (1)..(2): X is Dab
  MISC_FEATURE (4): X is Hdf
  MISC_FEATURE (5): X is Dab
  MISC_FEATURE (6)..(7): X is Hdf
  MISC_FEATURE (8)..(9): X is Dab
  MISC_FEATURE (12): X is Dab
  MISC_FEATURE (15): X is Dab
XXIXXXXXXPLXLLX

SEQ ID NO: 32 - protein, 15 aa, Artificial Sequence
  synthetic peptide
  MISC_FEATURE (1): N-terminal is lipidated by OctA
  MISC_FEATURE (1)..(2): X is Dab
  MISC_FEATURE (4): X is Hdf
  MISC_FEATURE (5): X is Dab
  MISC_FEATURE (6)..(7): X is Hdf
  MISC_FEATURE (8)..(9): X is Dab
  MISC_FEATURE (12): X is Dab
  MISC_FEATURE (15): X is Dab
XXLXXXXXXPLXLLX

SEQ ID NO: 33 - protein, 15 aa, Artificial Sequence
  synthetic peptide
  MISC_FEATURE (1): N-terminal is lipidated by OctA
  MISC_FEATURE (1)..(2): X is Dab
  MISC_FEATURE (4): X is Hdf
  MISC_FEATURE (5): X is Dab
  MISC_FEATURE (6)..(7): X is Hdf
  MISC_FEATURE (8)..(9): X is Dab
  MISC_FEATURE (12): X is Dab
  MISC_FEATURE (15): X is Dab
XXVXXXXXXPLXLLX

SEQ ID NO: 34 - protein, 15 aa, Artificial Sequence
  synthetic peptide
  MISC_FEATURE (1): N-terminal is lipidated by OctA
  MISC_FEATURE (1)..(2): X is Dab
  MISC_FEATURE (3): X is Hdf
  MISC_FEATURE (5): X is Dab
  MISC_FEATURE (6)..(7): X is Hdf
  MISC_FEATURE (8)..(9): X is Dab
  MISC_FEATURE (12): X is Dab
  MISC_FEATURE (15): X is Dab
XXXAXXXXXPLXLLX

SEQ ID NO: 35 - protein, 15 aa, Artificial Sequence
  synthetic peptide
  MISC_FEATURE (1): N-terminal is lipidated by OctA
  MISC_FEATURE (1)..(2): X is Dab
  MISC_FEATURE (3): X is Hdf
  MISC_FEATURE (5): X is Dab
  MISC_FEATURE (6)..(7): X is Hdf
  MISC_FEATURE (8)..(9): X is Dab
  MISC_FEATURE (12): X is Dab
  MISC_FEATURE (15): X is Dab
XXXFXXXXXPLXLLX

SEQ ID NO: 36 - protein, 15 aa, Artificial Sequence
  synthetic peptide
  MISC_FEATURE (1): N-terminal is lipidated by OctA
  MISC_FEATURE (1)..(2): X is Dab
  MISC_FEATURE (3): X is Hdf
  MISC_FEATURE (5): X is Dab
  MISC_FEATURE (6)..(7): X is Hdf
  MISC_FEATURE (8)..(9): X is Dab
  MISC_FEATURE (12): X is Dab
  MISC_FEATURE (15): X is Dab
XXXIXXXXXPLXLLX

SEQ ID NO: 37 - protein, 15 aa, Artificial Sequence
  synthetic peptide
  MISC_FEATURE (1): N-terminal is lipidated by OctA
  MISC_FEATURE (1)..(2): X is Dab
  MISC_FEATURE (3): X is Hdf
  MISC_FEATURE (5): X is Dab
  MISC_FEATURE (6)..(7): X is Hdf
  MISC_FEATURE (8)..(9): X is Dab
  MISC_FEATURE (12): X is Dab
  MISC_FEATURE (15): X is Dab
XXXLXXXXXPLXLLX

SEQ ID NO: 38 - protein, 15 aa, Artificial Sequence
  synthetic peptide
  MISC_FEATURE (1): N-terminal is lipidated by OctA
  MISC_FEATURE (1)..(2): X is Dab
  MISC_FEATURE (3): X is Hdf
  MISC_FEATURE (5): X is Dab
  MISC_FEATURE (6)..(7): X is Hdf
  MISC_FEATURE (8)..(9): X is Dab
  MISC_FEATURE (12): X is Dab
  MISC_FEATURE (15): X is Dab
XXXVXXXXXPLXLLX

SEQ ID NO: 39 - protein, 15 aa, Artificial Sequence
  synthetic peptide
  MISC_FEATURE (1): N-terminal is lipidated by OctA
  MISC_FEATURE (1)..(2): X is Dab
  MISC_FEATURE (3)..(4): X is Hdf
  MISC_FEATURE (5): X is Dab
  MISC_FEATURE (7): X is Hdf
  MISC_FEATURE (8)..(9): X is Dab
  MISC_FEATURE (12): X is Dab
  MISC_FEATURE (15): X is Dab
XXXXXAXXXPLXLLX

SEQ ID NO: 40 - protein, 15 aa, Artificial Sequence
  synthetic peptide
  MISC_FEATURE (1): N-terminal is lipidated by OctA
  MISC_FEATURE (1)..(2): X is Dab
  MISC_FEATURE (3)..(4): X is Hdf
  MISC_FEATURE (5): X is Dab
  MISC_FEATURE (7): X is Hdf
  MISC_FEATURE (8)..(9): X is Dab
  MISC_FEATURE (12): X is Dab
  MISC_FEATURE (15): X is Dab
XXXXXFXXXPLXLLX

SEQ ID NO: 41 - protein, 15 aa, Artificial Sequence
  synthetic peptide
  MISC_FEATURE (1): N-terminal is lipidated OctA
  MISC_FEATURE (1)..(2): X is Dab
  MISC_FEATURE (3)..(4): X is Hdf
  MISC_FEATURE (5): X is Dab
  MISC_FEATURE (7): X is Hdf
  MISC_FEATURE (8)..(9): X is Dab
  MISC_FEATURE (12): X is Dab
  MISC_FEATURE (15): X is Dab
XXXXXIXXXPLXLLX

SEQ ID NO: 42 - protein, 15 aa, Artificial Sequence
  synthetic peptide
  MISC_FEATURE (1): N-terminal is lipidated by OctA
  MISC_FEATURE (1)..(2): X is Dab
  MISC_FEATURE (3)..(4): X is Hdf
  MISC_FEATURE (5): X is Dab
  MISC_FEATURE (7): X is Hdf
  MISC_FEATURE (8)..(9): X is Dab
  MISC_FEATURE (12): X is Dab
  MISC_FEATURE (15): X is Dab
XXXXXLXXXPLXLLX

SEQ ID NO: 43 - protein, 15 aa, Artificial Sequence
  synthetic peptide
  MISC_FEATURE (1): N-terminal is lipidated by OctA
  MISC_FEATURE (1)..(2): X is Dab
  MISC_FEATURE (3)..(4): X is Hdf
  MISC_FEATURE (5): X is Dab
  MISC_FEATURE (7): X is Hdf
  MISC_FEATURE (8)..(9): X is Dab
  MISC_FEATURE (12): X is Dab
  MISC_FEATURE (15): X is Dab
XXXXXVXXXPLXLLX

SEQ ID NO: 44 - protein, 15 aa, Artificial Sequence
  synthetic peptide
  MISC_FEATURE (1): N-terminal is lipidated by OctA
  MISC_FEATURE (1)..(2): X is Dab
  MISC_FEATURE (3)..(4): X is Hdf
  MISC_FEATURE (5): X is Dab
  MISC_FEATURE (6): X is Hdf
  MISC_FEATURE (8)..(9): X is Dab
  MISC_FEATURE (12): X is Dab
  MISC_FEATURE (15): X is Dab
XXXXXXAXXPLXLLX

SEQ ID NO: 45 - protein, 15 aa, Artificial Sequence
  synthetic peptide
  MISC_FEATURE (1): N-terminal is lipidated by OctA
  MISC_FEATURE (1)..(2): X is Dab
  MISC_FEATURE (3)..(4): X is Hdf
  MISC_FEATURE (5): X is Dab
  MISC_FEATURE (6): X is Hdf
  MISC_FEATURE (8)..(9): X is Dab
  MISC_FEATURE (12): X is Dab
  MISC_FEATURE (15): X is Dab
XXXXXXFXXPLXLLX

SEQ ID NO: 46 - protein, 15 aa, Artificial Sequence
  synthetic peptide
  MISC_FEATURE (1): N-terminal is lipidated by OctA
  MISC_FEATURE (1)..(2): X is Dab
  MISC_FEATURE (3)..(4): X is Hdf
  MISC_FEATURE (5): X is Dab
  MISC_FEATURE (6): X is Hdf
  MISC_FEATURE (8)..(9): X is Dab
  MISC_FEATURE (12): X is Dab
  MISC_FEATURE (15): X is Dab
XXXXXXIXXPLXLLX

SEQ ID NO: 47 - protein, 15 aa, Artificial Sequence
  synthetic peptide
  MISC_FEATURE (1): N-terminal is lipidated by OctA
  MISC_FEATURE (1)..(2): X is Dab
  MISC_FEATURE (3)..(4): X is Hdf
  MISC_FEATURE (5): X is Dab
  MISC_FEATURE (6): X is Hdf
  MISC_FEATURE (8)..(9): X is Dab
  MISC_FEATURE (12): X is Dab
  MISC_FEATURE (15): X is Dab
XXXXXXLXXPLXLLX

SEQ ID NO: 48 - protein, 15 aa, Artificial Sequence
  synthetic peptide
  MISC_FEATURE (1): N-terminal is lipidated by OctA
  MISC_FEATURE (1)..(2): X is Dab
  MISC_FEATURE (3)..(4): X is Hdf
  MISC_FEATURE (5): X is Dab
  MISC_FEATURE (6): X is Hdf
  MISC_FEATURE (8)..(9): X is Dab
  MISC_FEATURE (12): X is Dab
  MISC_FEATURE (15): X is Dab
XXXXXXVXXPLXLLX

SEQ ID NO: 49 - protein, 15 aa, Artificial Sequence
  synthetic peptide
  MISC_FEATURE (1): N-terminal is lipidated by OctA
  MISC_FEATURE (1)..(2): X is Dab
  MISC_FEATURE (5): X is Dab
  MISC_FEATURE (8)..(9): X is Dab
  MISC_FEATURE (12): X is Dab
  MISC_FEATURE (15): X is Dab
XXAFXLAXXPLXLLX

SEQ ID NO: 50 - protein, 15 aa, Artificial Sequence
  synthetic peptide
  MISC_FEATURE (1): N-terminal is lipidated by OctA
  MISC_FEATURE (1)..(2): X is Dab
  MISC_FEATURE (5): X is Dab
  MISC_FEATURE (8)..(9): X is Dab
  MISC_FEATURE (12): X is Dab
  MISC_FEATURE (15): X is Dab
XXAFXVAXXPLXLLX

SEQ ID NO: 51 - protein, 15 aa, Artificial Sequence
  synthetic peptide
  MISC_FEATURE (1): N-terminal is lipidated by OctA
  MISC_FEATURE (1)..(2): X is Dab
  MISC_FEATURE (5): X is Dab
  MISC_FEATURE (8)..(9): X is Dab
  MISC_FEATURE (12): X is Dab
  MISC_FEATURE (15): X is Dab
XXAFXVVXXPLXLLX

SEQ ID NO: 52 - protein, 15 aa, Artificial Sequence
  synthetic peptide
  MISC_FEATURE (1): N-terminal is lipidated by OctA
  MISC_FEATURE (1)..(2): X is Dab
  MISC_FEATURE (5): X is Dab
  MISC_FEATURE (8)..(9): X is Dab
  MISC_FEATURE (12): X is Dab
  MISC_FEATURE (15): X is Dab
XXVFXVAXXPLXLLX

SEQ ID NO: 53 - protein, 15 aa, Artificial Sequence
  synthetic peptide
  MISC_FEATURE (1): N-terminal is lipidated by OctA
  MISC_FEATURE (2): X is Dab
  MISC_FEATURE (5): X is Dab
  MISC_FEATURE (8)..(9): X is Dab
  MISC_FEATURE (12): X is Dab
  MISC_FEATURE (15): X is Dab
SXALXLAXXPLXLLX

SEQ ID NO: 54 - protein, 15 aa, Artificial Sequence
  synthetic peptide
  MISC_FEATURE (1): N-terminal is lipidated by OctA
  MISC_FEATURE (1): X is Dab
  MISC_FEATURE (5): X is Dab
  MISC_FEATURE (8)..(9): X is Dab
  MISC_FEATURE (12): X is Dab
  MISC_FEATURE (15): X is Dab
XSALXLAXXPLXLLX

SEQ ID NO: 55 - protein, 15 aa, Artificial Sequence
  synthetic peptide
  MISC_FEATURE (1): N-terminal is lipidated by OctA
  MISC_FEATURE (1)..(2): X is Dab
  MISC_FEATURE (8)..(9): X is Dab
  MISC_FEATURE (12): X is Dab
  MISC_FEATURE (15): X is Dab
XXALSLAXXPLXLLX

SEQ ID NO: 56 - protein, 15 aa, Artificial Sequence
  synthetic peptide
  MISC_FEATURE (1)..(2): X is Dab
  MISC_FEATURE (5): X is Dab
  MISC_FEATURE (9): X is Dab
  MISC_FEATURE (12): X is Dab
  MISC_FEATURE (15): X is Dab
XXALXLASXPLXLLX

SEQ ID NO: 57 - protein, 15 aa, Artificial Sequence
  synthetic peptide
  MISC_FEATURE (1): N-terminal is lipidated by OctA
  MISC_FEATURE (1)..(2): X is Dab
  MISC_FEATURE (5): X is Dab
  MISC_FEATURE (8): X is Dab
  MISC_FEATURE (12): X is Dab
  MISC_FEATURE (15): X is Dab
XXALXLAXSPLXLLX

SEQ ID NO: 58 - protein, 15 aa, Artificial Sequence
  synthetic peptide
  MISC_FEATURE (1): N-terminal is lipidated by OctA
  MISC_FEATURE (1)..(2): X is Dab
  MISC_FEATURE (5): X is Dab
  MISC_FEATURE (8)..(9): X is Dab
  MISC_FEATURE (15): X is Dab
XXALXLAXXPLSLLX

SEQ ID NO: 59 - protein, 15 aa, Artificial Sequence
  synthetic peptide
  MISC_FEATURE (1): N-terminal is lipidated by OctA
  MISC_FEATURE (1)..(2): X is Dab
  MISC_FEATURE (5): X is Dab
  MISC_FEATURE (8)..(9): X is Dab
  MISC_FEATURE (12): X is Dab
XXALXLAXXPLXLLS

SEQ ID NO: 60 - protein, 15 aa, Artificial Sequence
  synthetic peptide
  MISC_FEATURE (1): N-terminal is lipidated by OctA
  MISC_FEATURE (1)..(2): X is Dab
  MISC_FEATURE (5): X is Dab
  MISC_FEATURE (8)..(9): X is Dab
  MISC_FEATURE (15): X is Dab
XXAFXVAXXPLSLLX

SEQ ID NO: 61 - protein, 15 aa, Artificial Sequence
  synthetic peptide
KKLLKLVKKPLKLLK

SEQ ID NO: 62 - protein, 15 aa, Artificial Sequence
  synthetic peptide
  MISC_FEATURE (1): N-terminal is lipidated by MyrA(myristic acid)
KKALKLAKKPLKLLK

SEQ ID NO: 63 - protein, 15 aa, Artificial Sequence
  synthetic peptide
  MISC_FEATURE (1): N-terminal is lipidated by PalA(palmitic acid)
KKALKLAKKPLKLLK

SEQ ID NO: 64 - protein, 15 aa, Artificial Sequence
  synthetic peptide
  MISC_FEATURE (1): N-terminal is lipidated by HexA
  MISC_FEATURE (1)..(2): X is Dab
  MISC_FEATURE (5): X is Dab
  MISC_FEATURE (8)..(9): X is Dab
  MISC_FEATURE (12): X is Dab
  MISC_FEATURE (15): X is Dab
XXALXLAXXPLXLLX

SEQ ID NO: 65 - protein, 15 aa, Artificial Sequence
  synthetic peptide
  MISC_FEATURE (1): N-terminal is lipidated by DecA
  MISC_FEATURE (1)..(2): X is Dab
  MISC_FEATURE (5): X is Dab
  MISC_FEATURE (8)..(9): X is Dab
  MISC_FEATURE (12): X is Dab
  MISC_FEATURE (15): X is Dab
XXALXLAXXPLXLLX

SEQ ID NO: 66 - protein, 15 aa, Artificial Sequence
  synthetic peptide
  MISC_FEATURE (1): N-terminal is lipidated by LauA
  MISC_FEATURE (1)..(2): X is Dab
  MISC_FEATURE (5): X is Dab
  MISC_FEATURE (8)..(9): X is Dab
  MISC_FEATURE (12): X is Dab
  MISC_FEATURE (15): X is Dab
XXALXLAXXPLXLLX

SEQ ID NO: 67 - protein, 15 aa, Artificial Sequence
  synthetic peptide
  MISC_FEATURE (1): N-terminal is lipidated by OctA
  MISC_FEATURE (1)..(2): X is Dab
  MISC_FEATURE (5): X is Dab
  MISC_FEATURE (8)..(9): X is Dab
XXALXLAXXPLSLLS